European Patent Application EP 4 130 028 A1, published February 8, 2023. Title: ENGINEERED TCR COMPLEX AND METHODS OF USING SAME. Applicant: Rhazes Therapeutics Ltd. The sequence listing filed with the application follows.

SEQUENCE LISTING (44 sequences)

SEQ ID NO: 1 - DNA, 20 bp, Artificial sequence
  gRNA
agagtctctcagctggtaca

SEQ ID NO: 2 - protein, 657 aa, Artificial sequence
  EGFP-P2A-TRAC(Cys,LVL)-P2A-TRBC1(Cys) amino acid sequence
MVSKGEELFTGVVPILVELDGDVNGHKFSVSGEGEGDATYGKLTLKFICTTGKLPVPWPTLVTTLTYGVQCFSRYPDHMKQHDFFKSAMPEGYVQERTIFFKDDGNYKTRAEVKFEGDTLVNRIELKGIDFKEDGNILGHKLEYNYNSHNVYIMADKQKNGIKVNFKIRHNIEDGSVQLADHYQQNTPIGDGPVLLPDNHYLSTQSALSKDPNEKRDHMVLLEFVTAAGITLGMDELYKATNFSLLKQAGDVEENPGPMALPVTALLLPLALLLHAARPIQNPDPAVYQLRDSKSSDKSVCLFTDFDSQTNVSQSKDSDVYITDKCVLDMRSMDFKSNSAVAWSNKSDFACANAFNNSIIPEDTFFPSPESSCDVKLVEKSFETDTNLNFQNLLVIVLRILLLKVAGFNLLMTLRLWSSRRKRGKPIPNPLLGLDSTSGSGATNFSLLKQAGDVEENPGPMALPVTALLLPLALLLHAARPDLNKVFPPEVAVFEPSEAEISHTQKATLVCLATGFFPDHVELSWWVNGKEVHSGVCTDPQPLKEQPALNDSRYCLSSRLRVSATFWQNPRNHFRCQVQFYGLSENDEWTQDRAKPVTQIVSAEAWGRADCGFTSVSYQQGVLSATILYEILLGKATLYAVLVSALVLMAMVKRKDF

SEQ ID NO: 3 - protein, 419 aa, Artificial sequence
  EGFP-P2A-TRAC amino acid sequence
MVSKGEELFTGVVPILVELDGDVNGHKFSVSGEGEGDATYGKLTLKFICTTGKLPVPWPTLVTTLTYGVQCFSRYPDHMKQHDFFKSAMPEGYVQERTIFFKDDGNYKTRAEVKFEGDTLVNRIELKGIDFKEDGNILGHKLEYNYNSHNVYIMADKQKNGIKVNFKIRHNIEDGSVQLADHYQQNTPIGDGPVLLPDNHYLSTQSALSKDPNEKRDHMVLLEFVTAAGITLGMDELYKATNFSLLKQAGDVEENPGPMALPVTALLLPLALLLHAARPIQNPDPAVYQLRDSKSSDKSVCLFTDFDSQTNVSQSKDSDVYITDKTVLDMRSMDFKSNSAVAWSNKSDFACANAFNNSIIPEDTFFPSPESSCDVKLVEKSFETDTNLNFQNLSVIGFRILLLKVAGFNLLMTLRLWSS

SEQ ID NO: 4 - protein, 182 aa, Homo sapiens
MEQGKGLAVLILAIILLQGTLAQSIKGNHLVKVYDYQEDGSVLLTCDAEAKNITWFKDGKMIGFLTEDKKKWNLGSNAKDPRGMYQCKGSQNKSKPLQVYYRMCQNCIELNAATISGFLFAEIVSIFVLAVGVYFIAGQDGVRQSRASDKQTLLPNDQLYQPLKDREDDQYSHLQGNQLRRN

SEQ ID NO: 5 - protein, 171 aa, Homo sapiens
MEHSTFLSGLVLATLLSQVSPFKIPIEELEDRVFVNCNTSITWVEGTVGTLLSDITRLDLGKRILDPRGIYRCNGTDIYKDKESTVQVHYRMCQSCVELDPATVAGIIVTDVIATLLLALGVFCFAGHETGRLSGAADTQALLRNDQVYQPLRDRDDAQYSHLGGNWARNK

SEQ ID NO: 6 - protein, 207 aa, Homo sapiens
MQSGTHWRVLGLCLLSVGVWGQDGNEEMGGITQTPYKVSISGTTVILTCPQYPGSEILWQHNDKNIGGDEDDKNIGSDEDHLSLKEFSELEQSGYYVCYPRGSKPEDANFYLYLRARVCENCMEMDVMSVATIVIVDICITGGLLLLVYYWSKNRKAKAKPVTRGAGAGGRQRGQNKERPPPVPNPDYEPIRKGQRDLYSGLNQRRI

SEQ ID NO: 7 - protein, 164 aa, Homo sapiens
MKWKALFTAAILQAQLPITEAQSFGLLDPKLCYLLDGILFIYGVILTALFLRVKFSRSADAPAYQQGQNQLYNELNLGRREEYDVLDKRRGRDPEMGGKPQRRKNPQEGLYNELQKDKMAEAYSEIGMKGERRRGKGHDGLYQGLSTATKDTYDALHMQALPPR

SEQ ID NO: 8 - protein, 136 aa, Mus musculus
IQNPEPAVYQLKDPRSQDSTLCLFTDFDSQINVPKTMESGTFITDKTVLDMKAMDSKSNGAIAWSNQTSFTCQDIFKETNATYPSSDVPCDATLTEKSFETDMNLNFQNLSVMGLRILLLKVAGFNLLMTLRLWSS

SEQ ID NO: 9 - protein, 140 aa, Homo sapiens
IQNPDPAVYQLRDSKSSDKSVCLFTDFDSQTNVSQSKDSDVYITDKTVLDMRSMDFKSNSAVAWSNKSDFACANAFNNSIIPEDTFFPSPESSCDVKLVEKSFETDTNLNFQNLSVIGFRILLLKVAGFNLLMTLRLWSS

SEQ ID NO: 10 - protein, 172 aa, Mus musculus
DLRNVTPPKVSLFEPSKAEIANKQKATLVCLARGFFPDHVELSWWVNGKEVHSGVSTDPQAYKESNYSYCLSSRLRVSATFWHNPRNHFRCQVQFHGLSEEDKWPEGSPKPVTQNISAEAWGRADCGITSASYQQGVLSATILYEILLGKATLYAVLVSTLVVMAMVKRKNS

SEQ ID NO: 11 - protein, 172 aa, Mus musculus
DLRNVTPPKVSLFEPSKAEIANKQKATLVCLARGFFPDHVELSWWVNGKEVHSGVSTDPQAYKESNYSYCLSSRLRVSATFWHNPRNHFRCQVQFHGLSEEDKWPEGSPKPVTQNISAEAWGRADCGITSASYHQGVLSATILYEILLGKATLYAVLVSGLVLMAMVKKKNS

SEQ ID NO: 12 - protein, 176 aa, Homo sapiens
DLNKVFPPEVAVFEPSEAEISHTQKATLVCLATGFFPDHVELSWWVNGKEVHSGVSTDPQPLKEQPALNDSRYCLSSRLRVSATFWQNPRNHFRCQVQFYGLSENDEWTQDRAKPVTQIVSAEAWGRADCGFTSVSYQQGVLSATILYEILLGKATLYAVLVSALVLMAMVKRKDF

SEQ ID NO: 13 - protein, 178 aa, Homo sapiens
DLKNVFPPKVAVFEPSEAEISHTQKATLVCLATGFYPDHVELSWWVNGKEVHSGVSTDPQPLKEQPALNDSRYCLSSRLRVSATFWQNPRNHFRCQVQFYGLSENDEWTQDRAKPVTQIVSAEAWGRADCGFTSESYQQGVLSATILYEILLGKATLYAVLVSALVLMAMVKRKDSRG

SEQ ID NO: 14 - protein, 140 aa, Artificial sequence
  amino acid sequence amino acid sequence
IQNPDPAVYQLRDSKSSDKSVCLFTDFDSQTNVSQSKDSDVYITDKTVLDMRSMDFKSNSAVAWSNKSDFACANAFNNSIIPEDTFFPSSDVPCDVKLVEKSFETDTNLNFQNLVVIGFRILLLKVAGFNLLMTLRLWSS

SEQ ID NO: 15 - protein, 176 aa, Artificial sequence
  mmTRBC1 amino acid sequence
DLNKVFPPEVAVFEPSKAEIAHTQKATLVCLATGFFPDHVELSWWVNGKEVHSGVSTDPQPLKEQPALNDSRYCLSSRLRVSATFWQNPRNHFRCQVQFYGLSENDEWTQDRAKPVTQIVSAEAWGRADCGITSASYHQGVLSATILYEILLGKATLYAVLVSALVLMAMVKRKDF

SEQ ID NO: 16 - protein, 178 aa, Artificial sequence
  mmTRBC2 amino acid sequence
DLKNVFPPKVAVFEPSKAEIAHTQKATLVCLATGFYPDHVELSWWVNGKEVHSGVSTDPQPLKEQPALNDSRYCLSSRLRVSATFWQNPRNHFRCQVQFYGLSENDEWTQDRAKPVTQIVSAEAWGRADCGITSASYHQGVLSATILYEILLGKATLYAVLVSALVLMAMVKRKDSRG

SEQ ID NO: 17 - protein, 140 aa, Artificial sequence
  TRAC (Cys) amino acid sequence
IQNPDPAVYQLRDSKSSDKSVCLFTDFDSQTNVSQSKDSDVYITDKCVLDMRSMDFKSNSAVAWSNKSDFACANAFNNSIIPEDTFFPSPESSCDVKLVEKSFETDTNLNFQNLSVIGFRILLLKVAGFNLLMTLRLWSS

SEQ ID NO: 18 - protein, 176 aa, Artificial sequence
  TRBC1(Cys) amino acid sequence
DLNKVFPPEVAVFEPSEAEISHTQKATLVCLATGFFPDHVELSWWVNGKEVHSGVCTDPQPLKEQPALNDSRYCLSSRLRVSATFWQNPRNHFRCQVQFYGLSENDEWTQDRAKPVTQIVSAEAWGRADCGFTSVSYQQGVLSATILYEILLGKATLYAVLVSALVLMAMVKRKDF

SEQ ID NO: 19 - protein, 178 aa, Artificial sequence
  TRBC2(Cys) amino acid sequence
DLKNVFPPKVAVFEPSEAEISHTQKATLVCLATGFYPDHVELSWWVNGKEVHSGVCTDPQPLKEQPALNDSRYCLSSRLRVSATFWQNPRNHFRCQVQFYGLSENDEWTQDRAKPVTQIVSAEAWGRADCGFTSESYQQGVLSATILYEILLGKATLYAVLVSALVLMAMVKRKDSRG

SEQ ID NO: 20 - protein, 140 aa, Artificial sequence
  TRAC (CYS,LVL) amino acid seaquence
IQNPDPAVYQLRDSKSSDKSVCLFTDFDSQTNVSQSKDSDVYITDKCVLDMRSMDFKSNSAVAWSNKSDFACANAFNNSIIPEDTFFPSPESSCDVKLVEKSFETDTNLNFQNLLVIVLRILLLKVAGFNLLMTLRLWSS

SEQ ID NO: 21 - protein, 140 aa, Artificial sequence
  mmTRAC (Cys) amino acid sequence
IQNPDPAVYQLRDSKSSDKSVCLFTDFDSQTNVSQSKDSDVYITDKCVLDMRSMDFKSNSAVAWSNKSDFACANAFNNSIIPEDTFFPSSDVPCDVKLVEKSFETDTNLNFQNLVVIGFRILLLKVAGFNLLMTLRLWSS

SEQ ID NO: 22 - protein, 140 aa, Artificial sequence
  mmTRAC (LVL) amino acid sequence
IQNPDPAVYQLRDSKSSDKSVCLFTDFDSQTNVSQSKDSDVYITDKTVLDMRSMDFKSNSAVAWSNKSDFACANAFNNSIIPEDTFFPSSDVPCDVKLVEKSFETDTNLNFQNLLVIVLRILLLKVAGFNLLMTLRLWSS

SEQ ID NO: 23 - protein, 140 aa, Artificial sequence
  mmTRAC (Cys, LVL) amino acid sequence
IQNPDPAVYQLRDSKSSDKSVCLFTDFDSQTNVSQSKDSDVYITDKCVLDMRSMDFKSNSAVAWSNKSDFACANAFNNSIIPEDTFFPSSDVPCDVKLVEKSFETDTNLNFQNLLVIVLRILLLKVAGFNLLMTLRLWSS

SEQ ID NO: 24 - protein, 176 aa, Artificial sequence
  mmTRBC1 (Cys) amino acid sequence
DLNKVFPPEVAVFEPSKAEIAHTQKATLVCLATGFFPDHVELSWWVNGKEVHSGVCTDPQPLKEQPALNDSRYCLSSRLRVSATFWQNPRNHFRCQVQFYGLSENDEWTQDRAKPVTQIVSAEAWGRADCGITSASYHQGVLSATILYEILLGKATLYAVLVSALVLMAMVKRKDF

SEQ ID NO: 25 - protein, 178 aa, Artificial sequence
  mmTRBC2 (Cys) amino acid sequence
DLKNVFPPKVAVFEPSKAEIAHTQKATLVCLATGFYPDHVELSWWVNGKEVHSGVCTDPQPLKEQPALNDSRYCLSSRLRVSATFWQNPRNHFRCQVQFYGLSENDEWTQDRAKPVTQIVSAEAWGRADCGITSASYHQGVLSATILYEILLGKATLYAVLVSALVLMAMVKRKDSRG

SEQ ID NO: 26 - protein, 635 aa, Artificial sequence
  EGFP-P2A-TRAC(Cys)-P2A-TRBC1(Cys) amino acid sequence
MVSKGEELFTGVVPILVELDGDVNGHKFSVSGEGEGDATYGKLTLKFICTTGKLPVPWPTLVTTLTYGVQCFSRYPDHMKQHDFFKSAMPEGYVQERTIFFKDDGNYKTRAEVKFEGDTLVNRIELKGIDFKEDGNILGHKLEYNYNSHNVYIMADKQKNGIKVNFKIRHNIEDGSVQLADHYQQNTPIGDGPVLLPDNHYLSTQSALSKDPNEKRDHMVLLEFVTAAGITLGMDELYKATNFSLLKQAGDVEENPGPMALPVTALLLPLALLLHAARPIQNPDPAVYQLRDSKSSDKSVCLFTDFDSQTNVSQSKDSDVYITDKCVLDMRSMDFKSNSAVAWSNKSDFACANAFNNSIIPEDTFFPSPESSCDVKLVEKSFETDTNLNFQNLSVIGFRILLLKVAGFNLLMTLRLWSSATNFSLLKQAGDVEENPGPMALPVTALLLPLALLLHAARPDLNKVFPPEVAVFEPSEAEISHTQKATLVCLATGFFPDHVELSWWVNGKEVHSGVCTDPQPLKEQPALNDSRYCLSSRLRVSATFWQNPRNHFRCQVQFYGLSENDEWTQDRAKPVTQIVSAEAWGRADCGFTSVSYQQGVLSATILYEILLGKATLYAVLVSALVLMAMVKRKDF

SEQ ID NO: 27 - protein, 657 aa, Artificial sequence
  EGFP-P2A-TRAC(Cys)-FurinV5P2A-TRBC1(Cys) amino acid sequence
MVSKGEELFTGVVPILVELDGDVNGHKFSVSGEGEGDATYGKLTLKFICTTGKLPVPWPTLVTTLTYGVQCFSRYPDHMKQHDFFKSAMPEGYVQERTIFFKDDGNYKTRAEVKFEGDTLVNRIELKGIDFKEDGNILGHKLEYNYNSHNVYIMADKQKNGIKVNFKIRHNIEDGSVQLADHYQQNTPIGDGPVLLPDNHYLSTQSALSKDPNEKRDHMVLLEFVTAAGITLGMDELYKATNFSLLKQAGDVEENPGPMALPVTALLLPLALLLHAARPIQNPDPAVYQLRDSKSSDKSVCLFTDFDSQTNVSQSKDSDVYITDKCVLDMRSMDFKSNSAVAWSNKSDFACANAFNNSIIPEDTFFPSPESSCDVKLVEKSFETDTNLNFQNLSVIGFRILLLKVAGFNLLMTLRLWSSRRKRGKPIPNPLLGLDSTSGSGATNFSLLKQAGDVEENPGPMALPVTALLLPLALLLHAARPDLNKVFPPEVAVFEPSEAEISHTQKATLVCLATGFFPDHVELSWWVNGKEVHSGVCTDPQPLKEQPALNDSRYCLSSRLRVSATFWQNPRNHFRCQVQFYGLSENDEWTQDRAKPVTQIVSAEAWGRADCGFTSVSYQQGVLSATILYEILLGKATLYAVLVSALVLMAMVKRKDF

SEQ ID NO: 28 - protein, 657 aa, Artificial sequence; identical to SEQ ID NO: 2
  EGFP-P2A-TRAC(Cys,LVL)-FurinV5P2A- TRBC1(Cys) amino acid sequence

SEQ ID NO: 29 - protein, 657 aa, Artificial sequence
  EGFP-P2A-mmTRAC-FurinV5P2A-mmTRBC1 amino acid sequence
MVSKGEELFTGVVPILVELDGDVNGHKFSVSGEGEGDATYGKLTLKFICTTGKLPVPWPTLVTTLTYGVQCFSRYPDHMKQHDFFKSAMPEGYVQERTIFFKDDGNYKTRAEVKFEGDTLVNRIELKGIDFKEDGNILGHKLEYNYNSHNVYIMADKQKNGIKVNFKIRHNIEDGSVQLADHYQQNTPIGDGPVLLPDNHYLSTQSALSKDPNEKRDHMVLLEFVTAAGITLGMDELYKATNFSLLKQAGDVEENPGPMALPVTALLLPLALLLHAARPIQNPDPAVYQLRDSKSSDKSVCLFTDFDSQTNVSQSKDSDVYITDKTVLDMRSMDFKSNSAVAWSNKSDFACANAFNNSIIPEDTFFPSSDVPCDVKLVEKSFETDTNLNFQNLSVIGFRILLLKVAGFNLLMTLRLWSSRRKRGKPIPNPLLGLDSTSGSGATNFSLLKQAGDVEENPGPMALPVTALLLPLALLLHAARPDLNKVFPPEVAVFEPSKAEIAHTQKATLVCLATGFFPDHVELSWWVNGKEVHSGVSTDPQPLKEQPALNDSRYCLSSRLRVSATFWQNPRNHFRCQVQFYGLSENDEWTQDRAKPVTQIVSAEAWGRADCGITSASYHQGVLSATILYEILLGKATLYAVLVSALVLMAMVKRKDF

SEQ ID NO: 30 - protein, 657 aa, Artificial sequence
  EGFP-P2A-mmTRAC(Cys)-FurinV5P2A-mmTRBC1(Cys) amino acid sequence
MVSKGEELFTGVVPILVELDGDVNGHKFSVSGEGEGDATYGKLTLKFICTTGKLPVPWPTLVTTLTYGVQCFSRYPDHMKQHDFFKSAMPEGYVQERTIFFKDDGNYKTRAEVKFEGDTLVNRIELKGIDFKEDGNILGHKLEYNYNSHNVYIMADKQKNGIKVNFKIRHNIEDGSVQLADHYQQNTPIGDGPVLLPDNHYLSTQSALSKDPNEKRDHMVLLEFVTAAGITLGMDELYKATNFSLLKQAGDVEENPGPMALPVTALLLPLALLLHAARPIQNPDPAVYQLRDSKSSDKSVCLFTDFDSQTNVSQSKDSDVYITDKCVLDMRSMDFKSNSAVAWSNKSDFACANAFNNSIIPEDTFFPSSDVPCDVKLVEKSFETDTNLNFQNLSVIGFRILLLKVAGFNLLMTLRLWSSRRKRGKPIPNPLLGLDSTSGSGATNFSLLKQAGDVEENPGPMALPVTALLLPLALLLHAARPDLNKVFPPEVAVFEPSKAEIAHTQKATLVCLATGFFPDHVELSWWVNGKEVHSGVCTDPQPLKEQPALNDSRYCLSSRLRVSATFWQNPRNHFRCQVQFYGLSENDEWTQDRAKPVTQIVSAEAWGRADCGITSASYHQGVLSATILYEILLGKATLYAVLVSALVLMAMVKRKDF

SEQ ID NO: 31 - protein, 657 aa, Artificial sequence
  EGFP-P2A-mmTRAC(LVL)-FurinV5P2A-mmTRBC1 amino acid sequence
MVSKGEELFTGVVPILVELDGDVNGHKFSVSGEGEGDATYGKLTLKFICTTGKLPVPWPTLVTTLTYGVQCFSRYPDHMKQHDFFKSAMPEGYVQERTIFFKDDGNYKTRAEVKFEGDTLVNRIELKGIDFKEDGNILGHKLEYNYNSHNVYIMADKQKNGIKVNFKIRHNIEDGSVQLADHYQQNTPIGDGPVLLPDNHYLSTQSALSKDPNEKRDHMVLLEFVTAAGITLGMDELYKATNFSLLKQAGDVEENPGPMALPVTALLLPLALLLHAARPIQNPDPAVYQLRDSKSSDKSVCLFTDFDSQTNVSQSKDSDVYITDKTVLDMRSMDFKSNSAVAWSNKSDFACANAFNNSIIPEDTFFPSSDVPCDVKLVEKSFETDTNLNFQNLLVIVLRILLLKVAGFNLLMTLRLWSSRRKRGKPIPNPLLGLDSTSGSGATNFSLLKQAGDVEENPGPMALPVTALLLPLALLLHAARPDLNKVFPPEVAVFEPSKAEIAHTQKATLVCLATGFFPDHVELSWWVNGKEVHSGVSTDPQPLKEQPALNDSRYCLSSRLRVSATFWQNPRNHFRCQVQFYGLSENDEWTQDRAKPVTQIVSAEAWGRADCGITSASYHQGVLSATILYEILLGKATLYAVLVSALVLMAMVKRKDF

SEQ ID NO: 32 - protein, 657 aa, Artificial sequence
  EGFP-P2A-mmTRAC(Cys,LVL)-FurinV5P2A-mmTRBC1(Cys) amino acid sequence
MVSKGEELFTGVVPILVELDGDVNGHKFSVSGEGEGDATYGKLTLKFICTTGKLPVPWPTLVTTLTYGVQCFSRYPDHMKQHDFFKSAMPEGYVQERTIFFKDDGNYKTRAEVKFEGDTLVNRIELKGIDFKEDGNILGHKLEYNYNSHNVYIMADKQKNGIKVNFKIRHNIEDGSVQLADHYQQNTPIGDGPVLLPDNHYLSTQSALSKDPNEKRDHMVLLEFVTAAGITLGMDELYKATNFSLLKQAGDVEENPGPMALPVTALLLPLALLLHAARPIQNPDPAVYQLRDSKSSDKSVCLFTDFDSQTNVSQSKDSDVYITDKCVLDMRSMDFKSNSAVAWSNKSDFACANAFNNSIIPEDTFFPSSDVPCDVKLVEKSFETDTNLNFQNLLVIVLRILLLKVAGFNLLMTLRLWSSRRKRGKPIPNPLLGLDSTSGSGATNFSLLKQAGDVEENPGPMALPVTALLLPLALLLHAARPDLNKVFPPEVAVFEPSKAEIAHTQKATLVCLATGFFPDHVELSWWVNGKEVHSGVCTDPQPLKEQPALNDSRYCLSSRLRVSATFWQNPRNHFRCQVQFYGLSENDEWTQDRAKPVTQIVSAEAWGRADCGITSASYHQGVLSATILYEILLGKATLYAVLVSALVLMAMVKRKDF

SEQ ID NO: 33 - DNA, 1908 bp, Artificial sequence
  EGFP-P2A-TRAC(Cys,LVL)-P2A-TRBC1(Cys) NA sequence
atggtgagcaagggcgaggagctgttcaccggggtggtgcccatcctggtcgagctggacggcgacgtaaacggccacaagttcagcgtgtccggcgagggcgagggcgatgccacctacggcaagctgaccctgaagttcatctgcaccaccggcaagctgcccgtgccctggcccaccctcgtgaccaccctgacctacggcgtgcagtgcttcagccgctaccccgaccacatgaagcagcacgacttcttcaagtccgccatgcccgaaggctacgtccaggagcgcaccatcttcttcaaggacgacggcaactacaagacccgcgccgaggtgaagttcgagggcgacaccctggtgaaccgcatcgagctgaagggcatcgacttcaaggaggacggcaacatcctggggcacaagctggagtacaactacaacagccacaacgtctatatcatggccgacaagcagaagaacggcatcaaggtgaacttcaagatccgccacaacatcgaggacggcagcgtgcagctcgccgaccactaccagcagaacacccccatcggcgacggccccgtgctgctgcccgacaaccactacctgagcacccagtccgccctgagcaaagaccccaacgagaagcgcgatcacatggtcctgctggagttcgtgaccgccgccgggatcactctcggcatggacgagctgtacaaggccacaaacttttctttgttgaaacaagccggagacgtagaggaaaacccaggtcctatggcactgccggtgaccgccttgctcctcccactcgctcttctcctccatgcggctcggcccatccagaacccagacccagcagtatatcagcttcgagattcaaagagttcagacaaatccgtatgtttgttcacagactttgattctcaaaccaatgtaagtcagtctaaagacagtgatgtctatataaccgataaatgcgtgctggacatgcggtcaatggacttcaagtccaacagcgcagttgcttggagcaacaaaagtgactttgcttgtgctaatgcgttcaacaactccataattccagaagatactttttttccgagtccggagtctagctgtgacgttaagttggtggagaaatcatttgagaccgacaccaatctgaatttccaaaatctgctggtaatagtactgaggattctgctgctcaaggtagctgggtttaaccttttgatgacgctccgactttggtcaagcgctacgaattttagtctcttgaaacaggccggtgatgtggaagaaaatcctggaccgatggcgttgcccgtaacggctttgcttcttcctcttgcattgctccttcatgcagcccggcccgacttgaacaaagtctttcctcctgaagtagctgtttttgagcccagtgaagcagagatttcacatacccaaaaggctacacttgtatgcctggctacgggtttcttccctgaccatgtggagctgagctggtgggtcaacggaaaggaggtacatagcggcgtctgcactgacccacagccactcaaagaacaacccgcattgaatgattcccggtactgtctctcatcacgactgcgcgtcagtgcgacgttctggcagaatcctcgaaatcactttaggtgccaagttcagttctatggtctctctgagaatgacgaatggactcaagatcgggccaaaccggttactcaaatcgttagtgcggaggcctggggccgcgcggattgtggcttcacttccgtaagttaccaacagggtgtgctgagcgcgaccatcctgtatgagatactgcttggcaaagcgacgctttacgccgttttggtgtcagcgttggtccttatggcgatggtcaaaaggaaggacttttag

SEQ ID NO: 34 - DNA, 1908 bp, Artificial sequence
  EGFP-P2A-TRAC(Cys,LVL)-P2A-TRBC1(Cys) NA sequence
atggtgagcaagggcgaggagctgttcaccggggtggtgcccatcctggtcgagctggacggcgacgtaaacggccacaagttcagcgtgtccggcgagggcgagggcgatgccacctacggcaagctgaccctgaagttcatctgcaccaccggcaagctgcccgtgccctggcccaccctcgtgaccaccctgacctacggcgtgcagtgcttcagccgctaccccgaccacatgaagcagcacgacttcttcaagtccgccatgcccgaaggctacgtccaggagcgcaccatcttcttcaaggacgacggcaactacaagacccgcgccgaggtgaagttcgagggcgacaccctggtgaaccgcatcgagctgaagggcatcgacttcaaggaggacggcaacatcctggggcacaagctggagtacaactacaacagccacaacgtctatatcatggccgacaagcagaagaacggcatcaaggtgaacttcaagatccgccacaacatcgaggacggcagcgtgcagctcgccgaccactaccagcagaacacccccatcggcgacggccccgtgctgctgcccgacaaccactacctgagcacccagtccgccctgagcaaagaccccaacgagaagcgcgatcacatggtcctgctggagttcgtgaccgccgccgggatcactctcggcatggacgagctgtacaaggccacaaacttttctttgttgaaacaagccggagacgtagaggaaaacccaggtcctatggcactgccggtgaccgccttgctcctcccactcgctcttctcctccatgcggctcggcccatccagaacccagacccagcagtatatcagcttcgagattcaaagagttcagacaaatccgtatgtttgttcacagactttgattctcaaaccaatgtaagtcagtctaaagacagtgatgtctatataaccgataaatgcgtgctggacatgcggtcaatggacttcaagtccaacagcgcagttgcttggagcaacaaaagtgactttgcttgtgctaatgcgttcaacaactccataattccagaagatactttttttccgagtccggagtctagctgtgacgttaagttggtggagaaatcatttgagaccgacaccaatctgaatttccaaaatctgtctgtaataggattcaggattctgctgctcaaggtagctgggtttaaccttttgatgacgctccgactttggtcaagcgctacgaattttagtctcttgaaacaggccggtgatgtggaagaaaatcctggaccgatggcgttgcccgtaacggctttgcttcttcctcttgcattgctccttcatgcagcccggcccgacttgaacaaagtctttcctcctgaagtagctgtttttgagcccagtgaagcagagatttcacatacccaaaaggctacacttgtatgcctggctacgggtttcttccctgaccatgtggagctgagctggtgggtcaacggaaaggaggtacatagcggcgtctgcactgacccacagccactcaaagaacaacccgcattgaatgattcccggtactgtctctcatcacgactgcgcgtcagtgcgacgttctggcagaatcctcgaaatcactttaggtgccaagttcagttctatggtctctctgagaatgacgaatggactcaagatcgggccaaaccggttactcaaatcgttagtgcggaggcctggggccgcgcggattgtggcttcacttccgtaagttaccaacagggtgtgctgagcgcgaccatcctgtatgagatactgcttggcaaagcgacgctttacgccgttttggtgtcagcgttggtccttatggcgatggtcaaaaggaaggacttttag

SEQ ID NO: 35 - DNA, 1974 bp, Artificial sequence
  EGFP-P2A-TRAC(Cys)-FurinV5P2A-TRBC1(Cys) NA sequence
atggtgagcaagggcgaggagctgttcaccggggtggtgcccatcctggtcgagctggacggcgacgtaaacggccacaagttcagcgtgtccggcgagggcgagggcgatgccacctacggcaagctgaccctgaagttcatctgcaccaccggcaagctgcccgtgccctggcccaccctcgtgaccaccctgacctacggcgtgcagtgcttcagccgctaccccgaccacatgaagcagcacgacttcttcaagtccgccatgcccgaaggctacgtccaggagcgcaccatcttcttcaaggacgacggcaactacaagacccgcgccgaggtgaagttcgagggcgacaccctggtgaaccgcatcgagctgaagggcatcgacttcaaggaggacggcaacatcctggggcacaagctggagtacaactacaacagccacaacgtctatatcatggccgacaagcagaagaacggcatcaaggtgaacttcaagatccgccacaacatcgaggacggcagcgtgcagctcgccgaccactaccagcagaacacccccatcggcgacggccccgtgctgctgcccgacaaccactacctgagcacccagtccgccctgagcaaagaccccaacgagaagcgcgatcacatggtcctgctggagttcgtgaccgccgccgggatcactctcggcatggacgagctgtacaaggccacaaacttttctttgttgaaacaagccggagacgtagaggaaaacccaggtcctatggcactgccggtgaccgccttgctcctcccactcgctcttctcctccatgcggctcggcccatccagaacccagacccagcagtatatcagcttcgagattcaaagagttcagacaaatccgtatgtttgttcacagactttgattctcaaaccaatgtaagtcagtctaaagacagtgatgtctatataaccgataaatgcgtgctggacatgcggtcaatggacttcaagtccaacagcgcagttgcttggagcaacaaaagtgactttgcttgtgctaatgcgttcaacaactccataattccagaagatactttttttccgagtccggagtctagctgtgacgttaagttggtggagaaatcatttgagaccgacaccaatctgaatttccaaaatctgtctgtaataggattcaggattctgctgctcaaggtagctgggtttaaccttttgatgacgctccgactttggtcaagccgacgaaaacgaggtaaaccaatcccaaacccgttgctgggtctggattctactagcggcagtggtgctacgaattttagtctcttgaaacaggccggtgatgtggaagaaaatcctggaccgatggcgttgcccgtaacggctttgcttcttcctcttgcattgctccttcatgcagcccggcccgacttgaacaaagtctttcctcctgaagtagctgtttttgagcccagtgaagcagagatttcacatacccaaaaggctacacttgtatgcctggctacgggtttcttccctgaccatgtggagctgagctggtgggtcaacggaaaggaggtacatagcggcgtctgcactgacccacagccactcaaagaacaacccgcattgaatgattcccggtactgtctctcatcacgactgcgcgtcagtgcgacgttctggcagaatcctcgaaatcactttaggtgccaagttcagttctatggtctctctgagaatgacgaatggactcaagatcgggccaaaccggttactcaaatcgttagtgcggaggcctggggccgcgcggattgtggcttcacttccgtaagttaccaacagggtgtgctgagcgcgaccatcctgtatgagatactgcttggcaaagcgacgctttacgccgttttggtgtcagcgttggtccttatggcgatggtcaaaaggaaggacttttag

SEQ ID NO: 36 - DNA, 1974 bp, Artificial sequence
  EGFP-P2A-TRAC(Cys,LVL)-FurinV5P2A- TRBC1(Cys) NA sequence
atggtgagcaagggcgaggagctgttcaccggggtggtgcccatcctggtcgagctggacggcgacgtaaacggccacaagttcagcgtgtccggcgagggcgagggcgatgccacctacggcaagctgaccctgaagttcatctgcaccaccggcaagctgcccgtgccctggcccaccctcgtgaccaccctgacctacggcgtgcagtgcttcagccgctaccccgaccacatgaagcagcacgacttcttcaagtccgccatgcccgaaggctacgtccaggagcgcaccatcttcttcaaggacgacggcaactacaagacccgcgccgaggtgaagttcgagggcgacaccctggtgaaccgcatcgagctgaagggcatcgacttcaaggaggacggcaacatcctggggcacaagctggagtacaactacaacagccacaacgtctatatcatggccgacaagcagaagaacggcatcaaggtgaacttcaagatccgccacaacatcgaggacggcagcgtgcagctcgccgaccactaccagcagaacacccccatcggcgacggccccgtgctgctgcccgacaaccactacctgagcacccagtccgccctgagcaaagaccccaacgagaagcgcgatcacatggtcctgctggagttcgtgaccgccgccgggatcactctcggcatggacgagctgtacaaggccacaaacttttctttgttgaaacaagccggagacgtagaggaaaacccaggtcctatggcactgccggtgaccgccttgctcctcccactcgctcttctcctccatgcggctcggcccatccagaacccagacccagcagtatatcagcttcgagattcaaagagttcagacaaatccgtatgtttgttcacagactttgattctcaaaccaatgtaagtcagtctaaagacagtgatgtctatataaccgataaatgcgtgctggacatgcggtcaatggacttcaagtccaacagcgcagttgcttggagcaacaaaagtgactttgcttgtgctaatgcgttcaacaactccataattccagaagatactttttttccgagtccggagtctagctgtgacgttaagttggtggagaaatcatttgagaccgacaccaatctgaatttccaaaatctgctggtaatagtactgaggattctgctgctcaaggtagctgggtttaaccttttgatgacgctccgactttggtcaagccgacgaaaacgaggtaaaccaatcccaaacccgttgctgggtctggattctactagcggcagtggtgctacgaattttagtctcttgaaacaggccggtgatgtggaagaaaatcctggaccgatggcgttgcccgtaacggctttgcttcttcctcttgcattgctccttcatgcagcccggcccgacttgaacaaagtctttcctcctgaagtagctgtttttgagcccagtgaagcagagatttcacatacccaaaaggctacacttgtatgcctggctacgggtttcttccctgaccatgtggagctgagctggtgggtcaacggaaaggaggtacatagcggcgtctgcactgacccacagccactcaaagaacaacccgcattgaatgattcccggtactgtctctcatcacgactgcgcgtcagtgcgacgttctggcagaatcctcgaaatcactttaggtgccaagttcagttctatggtctctctgagaatgacgaatggactcaagatcgggccaaaccggttactcaaatcgttagtgcggaggcctggggccgcgcggattgtggcttcacttccgtaagttaccaacagggtgtgctgagcgcgaccatcctgtatgagatactgcttggcaaagcgacgctttacgccgttttggtgtcagcgttggtccttatggcgatggtcaaaaggaaggacttttag

SEQ ID NO: 37 - DNA, 1974 bp, Artificial sequence
  EGFP-P2A-mmTRAC-FurinV5P2A-mmTRBC1 NA sequence
atggtgagcaagggcgaggagctgttcaccggggtggtgcccatcctggtcgagctggacggcgacgtaaacggccacaagttcagcgtgtccggcgagggcgagggcgatgccacctacggcaagctgaccctgaagttcatctgcaccaccggcaagctgcccgtgccctggcccaccctcgtgaccaccctgacctacggcgtgcagtgcttcagccgctaccccgaccacatgaagcagcacgacttcttcaagtccgccatgcccgaaggctacgtccaggagcgcaccatcttcttcaaggacgacggcaactacaagacccgcgccgaggtgaagttcgagggcgacaccctggtgaaccgcatcgagctgaagggcatcgacttcaaggaggacggcaacatcctggggcacaagctggagtacaactacaacagccacaacgtctatatcatggccgacaagcagaagaacggcatcaaggtgaacttcaagatccgccacaacatcgaggacggcagcgtgcagctcgccgaccactaccagcagaacacccccatcggcgacggccccgtgctgctgcccgacaaccactacctgagcacccagtccgccctgagcaaagaccccaacgagaagcgcgatcacatggtcctgctggagttcgtgaccgccgccgggatcactctcggcatggacgagctgtacaaggccacaaacttttctttgttgaaacaagccggagacgtagaggaaaacccaggtcctatggccctgccagttacggcattgttgcttcccttggctctcctcctccacgcagccagacctatacagaaccctgatccagcagtataccaattgcgggattcaaaaagcagcgataaaagtgtttgcttgttcacggacttcgattctcaaaccaacgttagtcaatcaaaagacagcgacgtatatatcacggataagacggttttggacatgagatctatggatttcaaatcaaactccgcagtagcttggtcaaacaaaagtgactttgcctgtgcaaatgcctttaacaatagtataattccagaggacactttctttcctagcagcgacgtcccctgtgatgtaaaattggtcgagaagagtttcgaaacagacacaaatctgaacttccagaatttgtctgtaataggattccgcattctccttctgaaagtagcaggctttaacctgttgatgactttgcggctgtggtcatctcgccgaaagcgagggaagcctattccaaatcctctcctcgggttggatagcacaagcgggtctggagcgacgaattttagtctgcttaagcaagctggggatgtagaagaaaatcctgggcctatggctctgccggttaccgcacttcttctcccgctcgcccttctccttcatgcggcgagacccgatctcaataaagtatttccacccgaagtcgcggtcttcgagccctcaaaagctgaaatcgctcacacgcaaaaagcaactttggtatgccttgctactggcttttttcccgatcatgtggaacttagttggtgggtgaatggtaaggaggttcattccggcgtatctactgacccgcagccccttaaggaacagcctgcactgaacgactctcgatactgcctgtcctcccgcttgcgagtaagtgcaactttttggcagaatcccaggaaccacttccggtgccaggttcagttttatggattgtccgaaaatgatgagtggacgcaagaccgagcaaagccagtcacacaaatcgtgtccgccgaagcctggggacgagcggactgcgggatcacgagcgcatcctatcatcaaggtgtactctcagcaaccatcctctacgagatattgctgggcaaagctaccttgtacgcggtgcttgtttctgcactggtgctgatggctatggtaaaacgcaaggacttctaa

SEQ ID NO: 38 - DNA, 1974 bp, Artificial sequence
  EGFP-P2A-mmTRAC(Cys)-FurinV5P2A-mmTRBC1(Cys) NA sequence
atggtgagcaagggcgaggagctgttcaccggggtggtgcccatcctggtcgagctggacggcgacgtaaacggccacaagttcagcgtgtccggcgagggcgagggcgatgccacctacggcaagctgaccctgaagttcatctgcaccaccggcaagctgcccgtgccctggcccaccctcgtgaccaccctgacctacggcgtgcagtgcttcagccgctaccccgaccacatgaagcagcacgacttcttcaagtccgccatgcccgaaggctacgtccaggagcgcaccatcttcttcaaggacgacggcaactacaagacccgcgccgaggtgaagttcgagggcgacaccctggtgaaccgcatcgagctgaagggcatcgacttcaaggaggacggcaacatcctggggcacaagctggagtacaactacaacagccacaacgtctatatcatggccgacaagcagaagaacggcatcaaggtgaacttcaagatccgccacaacatcgaggacggcagcgtgcagctcgccgaccactaccagcagaacacccccatcggcgacggccccgtgctgctgcccgacaaccactacctgagcacccagtccgccctgagcaaagaccccaacgagaagcgcgatcacatggtcctgctggagttcgtgaccgccgccgggatcactctcggcatggacgagctgtacaaggccacaaacttttctttgttgaaacaagccggagacgtagaggaaaacccaggtcctatggccctgccagttacggcattgttgcttcccttggctctcctcctccacgcagccagacctatacagaaccctgatccagcagtataccaattgcgggattcaaaaagcagcgataaaagtgtttgcttgttcacggacttcgattctcaaaccaacgttagtcaatcaaaagacagcgacgtatatatcacggataagtgcgttttggacatgagatctatggatttcaaatcaaactccgcagtagcttggtcaaacaaaagtgactttgcctgtgcaaatgcctttaacaatagtataattccagaggacactttctttcctagcagcgacgtcccctgtgatgtaaaattggtcgagaagagtttcgaaacagacacaaatctgaacttccagaatttgtctgtaataggattccgcattctccttctgaaagtagcaggctttaacctgttgatgactttgcggctgtggtcatctcgccgaaagcgagggaagcctattccaaatcctctcctcgggttggatagcacaagcgggtctggagcgacgaattttagtctgcttaagcaagctggggatgtagaagaaaatcctgggcctatggctctgccggttaccgcacttcttctcccgctcgcccttctccttcatgcggcgagacccgatctcaataaagtatttccacccgaagtcgcggtcttcgagccctcaaaagctgaaatcgctcacacgcaaaaagcaactttggtatgccttgctactggcttttttcccgatcatgtggaacttagttggtgggtgaatggtaaggaggttcattccggcgtatgcactgacccgcagccccttaaggaacagcctgcactgaacgactctcgatactgcctgtcctcccgcttgcgagtaagtgcaactttttggcagaatcccaggaaccacttccggtgccaggttcagttttatggattgtccgaaaatgatgagtggacgcaagaccgagcaaagccagtcacacaaatcgtgtccgccgaagcctggggacgagcggactgcgggatcacgagcgcatcctatcatcaaggtgtactctcagcaaccatcctctacgagatattgctgggcaaagctaccttgtacgcggtgcttgtttctgcactggtgctgatggctatggtaaaacgcaaggacttctaa

SEQ ID NO: 39 - DNA, 1974 bp, Artificial sequence
  EGFP-P2A-mmTRAC(LVL)-FurinV5P2A-mmTRBC1 NA sequence
atggtgagcaagggcgaggagctgttcaccggggtggtgcccatcctggtcgagctggacggcgacgtaaacggccacaagttcagcgtgtccggcgagggcgagggcgatgccacctacggcaagctgaccctgaagttcatctgcaccaccggcaagctgcccgtgccctggcccaccctcgtgaccaccctgacctacggcgtgcagtgcttcagccgctaccccgaccacatgaagcagcacgacttcttcaagtccgccatgcccgaaggctacgtccaggagcgcaccatcttcttcaaggacgacggcaactacaagacccgcgccgaggtgaagttcgagggcgacaccctggtgaaccgcatcgagctgaagggcatcgacttcaaggaggacggcaacatcctggggcacaagctggagtacaactacaacagccacaacgtctatatcatggccgacaagcagaagaacggcatcaaggtgaacttcaagatccgccacaacatcgaggacggcagcgtgcagctcgccgaccactaccagcagaacacccccatcggcgacggccccgtgctgctgcccgacaaccactacctgagcacccagtccgccctgagcaaagaccccaacgagaagcgcgatcacatggtcctgctggagttcgtgaccgccgccgggatcactctcggcatggacgagctgtacaaggccacaaacttttctttgttgaaacaagccggagacgtagaggaaaacccaggtcctatggccctgccagttacggcattgttgcttcccttggctctcctcctccacgcagccagacctatacagaaccctgatccagcagtataccaattgcgggattcaaaaagcagcgataaaagtgtttgcttgttcacggacttcgattctcaaaccaacgttagtcaatcaaaagacagcgacgtatatatcacggataagacggttttggacatgagatctatggatttcaaatcaaactccgcagtagcttggtcaaacaaaagtgactttgcctgtgcaaatgcctttaacaatagtataattccagaggacactttctttcctagcagcgacgtcccctgtgatgtaaaattggtcgagaagagtttcgaaacagacacaaatctgaacttccagaatttgcttgtaatagtgctgcgcattctccttctgaaagtagcaggctttaacctgttgatgactttgcggctgtggtcatctcgccgaaagcgagggaagcctattccaaatcctctcctcgggttggatagcacaagcgggtctggagcgacgaattttagtctgcttaagcaagctggggatgtagaagaaaatcctgggcctatggctctgccggttaccgcacttcttctcccgctcgcccttctccttcatgcggcgagacccgatctcaataaagtatttccacccgaagtcgcggtcttcgagccctcaaaagctgaaatcgctcacacgcaaaaagcaactttggtatgccttgctactggcttttttcccgatcatgtggaacttagttggtgggtgaatggtaaggaggttcattccggcgtatctactgacccgcagccccttaaggaacagcctgcactgaacgactctcgatactgcctgtcctcccgcttgcgagtaagtgcaactttttggcagaatcccaggaaccacttccggtgccaggttcagttttatggattgtccgaaaatgatgagtggacgcaagaccgagcaaagccagtcacacaaatcgtgtccgccgaagcctggggacgagcggactgcgggatcacgagcgcatcctatcatcaaggtgtactctcagcaaccatcctctacgagatattgctgggcaaagctaccttgtacgcggtgcttgtttctgcactggtgctgatggctatggtaaaacgcaaggacttctaa

SEQ ID NO: 40 - DNA, 1974 bp, Artificial sequence
  EGFP-P2A-mmTRAC(Cys,LVL)-FurinV5P2A-mmTRBC1(Cys) NA sequence
atggtgagcaagggcgaggagctgttcaccggggtggtgcccatcctggtcgagctggacggcgacgtaaacggccacaagttcagcgtgtccggcgagggcgagggcgatgccacctacggcaagctgaccctgaagttcatctgcaccaccggcaagctgcccgtgccctggcccaccctcgtgaccaccctgacctacggcgtgcagtgcttcagccgctaccccgaccacatgaagcagcacgacttcttcaagtccgccatgcccgaaggctacgtccaggagcgcaccatcttcttcaaggacgacggcaactacaagacccgcgccgaggtgaagttcgagggcgacaccctggtgaaccgcatcgagctgaagggcatcgacttcaaggaggacggcaacatcctggggcacaagctggagtacaactacaacagccacaacgtctatatcatggccgacaagcagaagaacggcatcaaggtgaacttcaagatccgccacaacatcgaggacggcagcgtgcagctcgccgaccactaccagcagaacacccccatcggcgacggccccgtgctgctgcccgacaaccactacctgagcacccagtccgccctgagcaaagaccccaacgagaagcgcgatcacatggtcctgctggagttcgtgaccgccgccgggatcactctcggcatggacgagctgtacaaggccacaaacttttctttgttgaaacaagccggagacgtagaggaaaacccaggtcctatggccctgccagttacggcattgttgcttcccttggctctcctcctccacgcagccagacctatacagaaccctgatccagcagtataccaattgcgggattcaaaaagcagcgataaaagtgtttgcttgttcacggacttcgattctcaaaccaacgttagtcaatcaaaagacagcgacgtatatatcacggataagtgcgttttggacatgagatctatggatttcaaatcaaactccgcagtagcttggtcaaacaaaagtgactttgcctgtgcaaatgcctttaacaatagtataattccagaggacactttctttcctagcagcgacgtcccctgtgatgtaaaattggtcgagaagagtttcgaaacagacacaaatctgaacttccagaatttgcttgtaatagtgctgcgcattctccttctgaaagtagcaggctttaacctgttgatgactttgcggctgtggtcatctcgccgaaagcgagggaagcctattccaaatcctctcctcgggttggatagcacaagcgggtctggagcgacgaattttagtctgcttaagcaagctggggatgtagaagaaaatcctgggcctatggctctgccggttaccgcacttcttctcccgctcgcccttctccttcatgcggcgagacccgatctcaataaagtatttccacccgaagtcgcggtcttcgagccctcaaaagctgaaatcgctcacacgcaaaaagcaactttggtatgccttgctactggcttttttcccgatcatgtggaacttagttggtgggtgaatggtaaggaggttcattccggcgtatgcactgacccgcagccccttaaggaacagcctgcactgaacgactctcgatactgcctgtcctcccgcttgcgagtaagtgcaactttttggcagaatcccaggaaccacttccggtgccaggttcagttttatggattgtccgaaaatgatgagtggacgcaagaccgagcaaagccagtcacacaaatcgtgtccgccgaagcctggggacgagcggactgcgggatcacgagcgcatcctatcatcaaggtgtactctcagcaaccatcctctacgagatattgctgggcaaagctaccttgtacgcggtgcttgtttctgcactggtgctgatggctatggtaaaacgcaaggacttctaa

SEQ ID NO: 41 - DNA, 1260 bp, Artificial sequence
  EGFP-P2A-TRAC NA sequence
atggtgagcaagggcgaggagctgttcaccggggtggtgcccatcctggtcgagctggacggcgacgtaaacggccacaagttcagcgtgtccggcgagggcgagggcgatgccacctacggcaagctgaccctgaagttcatctgcaccaccggcaagctgcccgtgccctggcccaccctcgtgaccaccctgacctacggcgtgcagtgcttcagccgctaccccgaccacatgaagcagcacgacttcttcaagtccgccatgcccgaaggctacgtccaggagcgcaccatcttcttcaaggacgacggcaactacaagacccgcgccgaggtgaagttcgagggcgacaccctggtgaaccgcatcgagctgaagggcatcgacttcaaggaggacggcaacatcctggggcacaagctggagtacaactacaacagccacaacgtctatatcatggccgacaagcagaagaacggcatcaaggtgaacttcaagatccgccacaacatcgaggacggcagcgtgcagctcgccgaccactaccagcagaacacccccatcggcgacggccccgtgctgctgcccgacaaccactacctgagcacccagtccgccctgagcaaagaccccaacgagaagcgcgatcacatggtcctgctggagttcgtgaccgccgccgggatcactctcggcatggacgagctgtacaaggccacaaacttttctttgttgaaacaagccggagacgtagaggaaaacccaggtcctatggcactgccggtgaccgccttgctcctcccactcgctcttctcctccatgcggctcggcccatccagaacccagacccagcagtatatcagcttcgagattcaaagagttcagacaaatccgtatgtttgttcacagactttgattctcaaaccaatgtaagtcagtctaaagacagtgatgtctatataaccgataaaactgtgctggacatgcggtcaatggacttcaagtccaacagcgcagttgcttggagcaacaaaagtgactttgcttgtgctaatgcgttcaacaactccataattccagaagatactttttttccgagtccggagtctagctgtgacgttaagttggtggagaaatcatttgagaccgacaccaatctgaatttccaaaatctgtctgtaataggattcaggattctgctgctcaaggtagctgggtttaaccttttgatgacgctccgactttggtcaagctag

SEQ ID NO: 42 - protein, 21 aa, Artificial sequence
  CD8 membrane trafficking signal (AA sequence)
MALPVTALLLPLALLLHAARP

SEQ ID NO: 43 - DNA, 63 bp, Artificial sequence
  CD8 membrane trafficking signal (NA sequence)
atggcactgccggtgaccgccttgctcctcccactcgctcttctcctccatgcggctcggccc

SEQ ID NO: 44 - protein, 140 aa, Artificial sequence
  TRAC (LVL)
IQNPDPAVYQLRDSKSSDKSVCLFTDFDSQTNVSQSKDSDVYITDKTVLDMRSMDFKSNSAVAWSNKSDFACANAFNNSIIPEDTFFPSPESSCDVKLVEKSFETDTNLNFQNLLVIVLRILLLKVAGFNLLMTLRLWSS